European Patent Application EP 4 186 499 A1, published May 31, 2023. Title: OPHTHALMIC COMPOSITIONS FOR TREATMENT OF CORNEAL LESIONS. Applicant: PROFESSIONAL DIETETICS SPA. The sequence listing filed with the application follows.

SEQUENCE LISTING (6 sequences)

SEQ ID NO: 1 - DNA, 21 bp, synthetic construct
  source 1..21: mol_type = other DNA
ccttgcttgcttcggctaaaa

SEQ ID NO: 2 - DNA, 20 bp, synthetic construct
  source 1..20: mol_type = other DNA
ctgctgcattgagctttgct

SEQ ID NO: 3 - DNA, 20 bp, synthetic construct
  source 1..20: mol_type = other DNA
tcgggaacaagggctaaagg

SEQ ID NO: 4 - DNA, 20 bp, synthetic construct
  source 1..20: mol_type = other DNA
cccgtgatcagtgggttcat

SEQ ID NO: 5 - DNA, 20 bp, synthetic construct
  source 1..20: mol_type = other DNA
acagaagccgacagcagaat

SEQ ID NO: 6 - DNA, 20 bp, synthetic construct
  source 1..20: mol_type = other DNA
gcacaggaaagcaaagtcag